European Patent Application EP 4 375 292 A1, published May 29, 2024. Title: Novel Chimeric Antigen Receptor and Immune Cell Expressing the Same. Applicant: KOREA RESEARCH INSTITUTE OF BIOSCIENCE AND BIOTECHNOLOGY. The sequence listing filed with the application follows.

SEQUENCE LISTING (13 sequences)

SEQ ID NO: 1 - protein, 155 aa, synthetic construct
  REGION 1..155: note = P75NTR intracellular domain
KRWNSCKQNKQGANSRPVNQTPPPEGEKLHSDSGISVDSQSLHDQQPHTQTASGQALKGDGGLYSSLPPAKREEVEKLLNGSAGDTWRHLAGELGYQPEHIDSFTHEACPVRALLASWATQDSATLDALLAALRRIQRADLVESLCSESTATSPV

SEQ ID NO: 2 - DNA, 468 bp, synthetic construct
  misc_feature 1..468: note = P75NTR intracellular domain
  source 1..468: mol_type = other DNA
aagaggtggaacagctgcaagcagaacaagcaaggagccaacagccggccagtgaaccagacgcccccaccagagggagaaaaactccacagcgacagtggcatctccgtggacagccagagcctgcatgaccagcagccccacacgcagacagcctcgggccaggccctcaagggtgacggaggcctctacagcagcctgcccccagccaagcgggaggaggtggagaagcttctcaacggctctgcgggggacacctggcggcacctggcgggcgagctgggctaccagcccgagcacatagactcctttacccatgaggcctgccccgttcgcgccctgcttgcaagctgggccacccaggacagcgccacactggacgccctcctggccgccctgcgccgcatccagcgagccgacctcgtggagagtctgtgcagtgagtccactgccacatccccggtgtaa

SEQ ID NO: 3 - protein, 243 aa, synthetic construct
  REGION 1..243: note = EGFR scFv
EVQLVESGGGLVQPGGSLRLSCAASGFTFSSYEMSWVRQAPGKGLEWVSAISGSGSNTYYADSVKGRFTISRDNSKNTLYLQMNSLRAEDTAVYYCAKESELEYWGAFDHWGQGTLVTVSSGGGGSGGGGSGGGGSDIQMTQSPSSLSASVGDRVTITCRASQSISNYLNWYQQKPGKAPKLLIYDASNLHSGVPSRFSGSGSGTDFTLTISSLQPEDFATYYCQQSHTFPWTFGQGTKVEIK

SEQ ID NO: 4 - DNA, 729 bp, synthetic construct
  misc_feature 1..729: note = EGFR scFv
  source 1..729: mol_type = other DNA
gaagtacagttggtcgaaagtggcggtggcctcgtgcaaccgggtggttcactgcgtctgagctgcgccgcctcgggttttactttctcttcttatgaaatgtcttgggttcgtcaggcgccgggcaagggtctcgaatgggtttcagcaatctctggttctggttctaatacttactatgccgattcagtgaagggtcgctttaccatttcccgtgacaactctaagaatactctgtatctgcagatgaactcgctgcgtgccgaagacacggccgtctattattgcgccaaagaatctgaactggaatactggggtgcattcgatcattggggtcagggcactttagtgaccgtctcatcgggtggaggcggttcaggcggaggtggatccggcggtggcggatcggacattcaaatgacgcagagtccctcctcactgagtgctagcgtgggcgatcgtgtgacaattacttgtcgcgctagccagtctatctctaattacctgaactggtatcagcagaaaccgggcaaggcgccaaaattgctgatttacgatgcatccaatctgcactctggtgtaccgtcccgtttctctggcagcggttctggtacggattttaccctgaccatctcaagcctccagcctgaagattttgccacctattattgtcagcaatctcacacttttccgtggacgttcgggcagggaactaaagtggaaattaaa

SEQ ID NO: 5 - protein, 10 aa, synthetic construct
  REGION 1..10: note = Myc epitope
EQKLISEEDL

SEQ ID NO: 6 - DNA, 30 bp, synthetic construct
  misc_feature 1..30: note = Myc epitope
  source 1..30: mol_type = other DNA
gaacaaaaactcatctcagaagaggatctg

SEQ ID NO: 7 - protein, 68 aa, synthetic construct
  REGION 1..68: note = CD8 hinge domain
GVTVSSALSNSIMYFSHFVPVFLPAKPTTTPAPRPPTPAPTIASQPLSLRPEACRPAAGGAVHTRGLD

SEQ ID NO: 8 - DNA, 204 bp, synthetic construct
  misc_feature 1..204: note = CD8 hinge domain
  source 1..204: mol_type = other DNA
ggggtcaccgtctcttcagcgctgagcaactccatcatgtacttcagccacttcgtgccggtcttcctgccagcgaagcccaccacgacgccagcgccgcgaccaccaacaccggcgcccaccatcgcgtcgcagcccctgtccctgcgcccagaggcatgccggccagcggcggggggcgcagtgcacacgagggggctggat

SEQ ID NO: 9 - protein, 21 aa, synthetic construct
  REGION 1..21: note = signal peptide
MALPVTALLLPLALLLHAARP

SEQ ID NO: 10 - DNA, 65 bp, synthetic construct
  misc_feature 1..65: note = signal peptide
  source 1..65: mol_type = other DNA
atggccttaccagtgaccgccttgctcctgccgctggccttactgctccacgccgccaggccggc

SEQ ID NO: 11 - protein, 28 aa, synthetic construct
  REGION 1..28: note = transmembrane domain
PFWVLVVVGGVLACYSLLVTVAFIIFWV

SEQ ID NO: 12 - DNA, 84 bp, synthetic construct
  misc_feature 1..84: note = transmembrane domain
  source 1..84: mol_type = other DNA
cccttttgggtgctggtggtggttggtggagtcctggcttgctatagcttgctagtaacagtggcctttattattttctgggtg

SEQ ID NO: 13 - DNA, 1546 bp, synthetic construct
  misc_feature 1..1546: note = P75NTR CAR
  source 1..1546: mol_type = other DNA
gaagtacagttggtcgaaagtggcggtggcctcgtgcaaccgggtggttcactgcgtctgagctgcgccgcctcgggttttactttctcttcttatgaaatgtcttgggttcgtcaggcgccgggcaagggtctcgaatgggtttcagcaatctctggttctggttctaatacttactatgccgattcagtgaagggtcgctttaccatttcccgtgacaactctaagaatactctgtatctgcagatgaactcgctgcgtgccgaagacacggccgtctattattgcgccaaagaatctgaactggaatactggggtgcattcgatcattggggtcagggcactttagtgaccgtctcatcgggtggaggcggttcaggcggaggtggatccggcggtggcggatcggacattcaaatgacgcagagtccctcctcactgagtgctagcgtgggcgatcgtgtgacaattacttgtcgcgctagccagtctatctctaattacctgaactggtatcagcagaaaccgggcaaggcgccaaaattgctgatttacgatgcatccaatctgcactctggtgtaccgtcccgtttctctggcagcggttctggtacggattttaccctgaccatctcaagcctccagcctgaagattttgccacctattattgtcagcaatctcacacttttccgtggacgttcgggcagggaactaaagtggaaattaaaggcccgggaggccgaacaaaaactcatctcagaagaggatctgaaacttggggtcaccgtctcttcagcgctgagcaactccatcatgtacttcagccacttcgtgccggtcttcctgccagcgaagcccaccacgacgccagcgccgcgaccaccaacaccggcgcccaccatcgcgtcgcagcccctgtccctgcgcccagaggcatgccggccagcggcggggggcgcagtgcacacgagggggctggataagcttcccttttgggtgctggtggtggttggtggagtcctggcttgctatagcttgctagtaacagtggcctttattattttctgggtggaattcaagaggtggaacagctgcaagcagaacaagcaaggagccaacagccggccagtgaaccagacgcccccaccagagggagaaaaactccacagcgacagtggcatctccgtggacagccagagcctgcatgaccagcagccccacacgcagacagcctcgggccaggccctcaagggtgacggaggcctctacagcagcctgcccccagccaagcgggaggaggtggagaagcttctcaacggctctgcgggggacacctggcggcacctggcgggcgagctgggctaccagcccgagcacatagactcctttacccatgaggcctgccccgttcgcgccctgcttgcaagctgggccacccaggacagcgccacactggacgccctcctggccgccctgcgccgcatccagcgagccgacctcgtggagagtctgtgcagtgagtccactgccacatccccggtgtaa